European Patent Specification EP 3 943 608 B1, published July 12, 2023. Title: METHOD OF DETECTING AN ENDOTOXIN USING LIMULUS AMEBOCYTE LYSATE SUBSTANTIALLY FREE OF COAGULOGEN. Applicant: LONZA WALKERSVILLE, INC. Application PCT/US2017/045137. The sequence listing filed with the application follows.

SEQUENCE LISTING (4 sequences)

SEQ ID NO: 1 - protein, 4 aa, Artificial Sequence
  Description of Artificial Sequence: Synthetic peptide
  N-term Ac
  C-term pNA
IEAR

SEQ ID NO: 2 - protein, 10 aa, Limulus polyphemus
GDPNVPTCLC

SEQ ID NO: 3 - protein, 10 aa, Limulus polyphemus
KVIVSQEKTD

SEQ ID NO: 4 - protein, 10 aa, Limulus polyphemus
GFSIFGGHPA